European Patent Specification EP 4 326 882 B1, published January 14, 2026. Title: Methods and means for the prevention and/or treatment of joint damage in hemophilia. Applicant: uniQure N.V. The sequence listing filed with the application follows.

SEQUENCE LISTING (1 sequence)

SEQ ID NO: 1 - protein, 415 aa, human
  MISC_FEATURE (86)..(86): Xaa can be V(wt) or A
  MISC_FEATURE (148)..(148): Xaa can be A(wt) or T(wt)
  MISC_FEATURE (277)..(277): Xaa can be E(wt) or A
  MISC_FEATURE (318)..(318): Xaa can be R(wt) or Y
  MISC_FEATURE (338)..(338): Xaa can be R(wt) or L or Q or E or A
  MISC_FEATURE (343)..(343): Xaa can be T(wt) or R
YNSGKLEEFVQGNLERECMEEKCSFEEAREVFENTERTTEFWKQYVDGDQCESNPCLNGGSCKDDINSYECWCPFGFEGKNCELDXTCNIKNGRCEQFCKNSADNKVVCSCTEGYRLAENQKSCEPAVPFPCGRVSVSQTSKLTRAEXVFPDVDYVNSTEAETILDNITQSTQSFNDFTRVVGGEDAKPGQFPWQVVLNGKVDAFCGGSIVNEKWIVTAAHCVETGVKITVVAGEHNIEETEHTEQKRNVIRIIPHHNYNAAINKYNHDIALLELDXPLVLNSYVTPICIADKEYTNIFLKFGSGYVSGWGRVFHKGXSALVLQYLRVPLVDRATCLXSTKFXIYNNMFCAGFHEGGRDSCQGDSGGPHVTEVEGTSFLTGIISWGEECAMKGKYGIYTKVSRYVNWIKEKTKLT